European Patent Application EP 4 176 884 A1, published May 10, 2023. Title: Methods of Promoting Bone Growth by Administration of Sost Antagonist. Applicant: Ossifi-Mab LLC. The sequence listing filed with the application follows.

SEQUENCE LISTING (23 sequences)

SEQ ID NO: 1 - protein, 11 aa, Homo sapiens
DTGTDRIEVTR

SEQ ID NO: 2 - protein, 14 aa, Homo sapiens
ENNKTMNRAENGGR

SEQ ID NO: 3 - protein, 16 aa, Homo sapiens
HPFETKDVSEYSCREL

SEQ ID NO: 4 - protein, 17 aa, Homo sapiens
RELHFTRYVTDGPCRSA

SEQ ID NO: 5 - protein, 17 aa, Homo sapiens
QLLCPGGEAPRARKVRL

SEQ ID NO: 6 - protein, 14 aa, Canis lupus
ENNKTMNRAENGGR

SEQ ID NO: 7 - protein, 14 aa, Canis lupus
HPFETKSEYSCREL

SEQ ID NO: 8 - protein, 17 aa, Canis lupus
RELHFTRYVTDGPCRSA

SEQ ID NO: 9 - protein, 17 aa, Canis lupus
RVQLLCPGGAAPRARKV

SEQ ID NO: 10 - protein, 14 aa, Pan troglodytes
ENNKTMNRAENGGR

SEQ ID NO: 11 - protein, 16 aa, Pan troglodytes
HPFETKDVSEYSCREL

SEQ ID NO: 12 - protein, 17 aa, Pan troglodytes
RELHFTRYVTDGPCRSA

SEQ ID NO: 13 - protein, 15 aa, Pan troglodytes
LCPGGAAPRARKVRL

SEQ ID NO: 14 - protein, 14 aa, Homo sapiens
SSNSTLNQARNGGR

SEQ ID NO: 15 - protein, 16 aa, Homo sapiens
TGLDRNSRVQVGCREL

SEQ ID NO: 16 - protein, 16 aa, Mus musculus
TGLDRNTRVQVGCREL

SEQ ID NO: 17 - protein, 17 aa, Homo sapiens
RELRSTKYISDGQCTSI

SEQ ID NO: 18 - protein, 16 aa, Homo sapiens
QLQCQDGSTRTYKITV

SEQ ID NO: 19 - protein, 15 aa, Homo sapiens
PLKELVCAGECLPLP

SEQ ID NO: 20 - protein, 14 aa, Homo sapiens
GTKYWSRRSSQEWR

SEQ ID NO: 21 - protein, 14 aa, Homo sapiens
CKCKRYTRQHNESS

SEQ ID NO: 22 - protein, 213 aa, Homo sapiens
MQLPLALCLVCLLVHTAFRVVEGQGWQAFKNDATEIIPELGEYPEPPPELENNKTMNRAENGGRPPHHPFETKDVSEYSCRELHFTRYVTDGPCRSAKPVTELVCSGQCGPARLLPNAIGRGKWWRPSGPDFRCIPDRYRAQRVQLLCPGGEAPRARKVRLVASCKCKRLTRFHNQSELKDFGTEAARPQKGRKPRPRARSAKANQAELENAY

SEQ ID NO: 23 - protein, 15 aa, Homo sapiens
PVTELVCSGQCGPAR